European Patent Application EP 4 541 811 A1, published April 23, 2025. Title: T CELL RECEPTOR TARGETING KRAS G12V MUTANT POLYPEPTIDE, AND USE THEREOF. Applicant: IMMUXELL BIOTECH LTD. Application EP EP23823090.8, filed June 12, 2023. The sequence listing filed with the application follows.

SEQUENCE LISTING (30 sequences)

SEQ ID NO: 1 - protein, 17 aa, Homo sapiens
CAVRDIEGAGNNRKLIW

SEQ ID NO: 2 - protein, 14 aa, Homo sapiens
CASSEGQYSYEQYF

SEQ ID NO: 3 - protein, 6 aa, Homo sapiens
SVSGNP

SEQ ID NO: 4 - protein, 6 aa, Homo sapiens
YITGDN

SEQ ID NO: 5 - protein, 5 aa, Homo sapiens
SNHLY

SEQ ID NO: 6 - protein, 6 aa, Homo sapiens
FYNNEI

SEQ ID NO: 7 - protein, 136 aa, Homo sapiens
MASAPISMLAMLFTLSGLRAQSVAQPEDQVNVAEGNPLTVKCTYSVSGNPYLFWYVQYPNRGLQFLLKYITGDNLVKGSYGFEAEFNKSQTSFHLKKPSALVSDSALYFCAVRDIEGAGNNRKLIWGLGTSLAVNP

SEQ ID NO: 8 - protein, 133 aa, Homo sapiens
MDTWLVCWAIFSLLKAGLTEPEVTQTPSHQVTQMGQEVILRCVPISNHLYFYWYRQILGQKVEFLVSFYNNEISEKSEIFDDQFSVERPDGSNFTLKIRSTKLEDSAMYFCASSEGQYSYEQYFGPGTRLTVT

SEQ ID NO: 9 - protein, 137 aa, Mus musculus
NIQNPEPAVYQLKDPRSQDSTLCLFTDFDSQINVPKTMESGTFITDKCVLDMKAMDSKSNGAIAWSNQTSFTCQDIFKETNATYPSSDVPCDATLTEKSFETDMNLNFQNLLVIVLRILLLKVAGFNLLMTLRLWSS

SEQ ID NO: 10 - protein, 173 aa, Mus musculus
EDLRNVTPPKVSLFEPSKAEIANKQKATLVCLARGFFPDHVELSWWVNGKEVHSGVCTDPQAYKESNYSYCLSSRLRVSATFWHNPRNHFRCQVQFHGLSEEDKWPEGSPKPVTQNISAEAWGRADCGITSASYQQGVLSATILYEILLGKATLYAVLVSTLVVMAMVKRKNS

SEQ ID NO: 11 - DNA, 408 bp, Homo sapiens
  source 1..408: mol_type = genomic DNA
atggcctctgcacccatctcgatgcttgcgatgctcttcacattgagtgggctgagagctcagtcagtggctcagccggaagatcaggtcaacgttgctgaagggaatcctctgactgtgaaatgcacctattcagtctctggaaacccttatcttttttggtatgttcaataccccaaccgaggcctccagttccttctgaaatacatcacaggggataacctggttaaaggcagctatggctttgaagctgaatttaacaagagccaaacctccttccacctgaagaaaccatctgcccttgtgagcgactccgctttgtacttctgtgctgtgagagacattgagggtgctggcaacaaccgtaagctgatttggggattgggaacaagcctggcagtaaatccg

SEQ ID NO: 12 - DNA, 399 bp, Homo sapiens
  source 1..399: mol_type = genomic DNA
atggatacctggctcgtatgctgggcaatttttagtctcttgaaagcaggactcacagaacctgaagtcacccagactcccagccatcaggtcacacagatgggacaggaagtgatcttgcgctgtgtccccatctctaatcacttatacttctattggtacagacaaatcttggggcagaaagtcgagtttctggtttccttttataataatgaaatctcagagaagtctgaaatattcgatgatcaattctcagttgaaaggcctgatggatcaaatttcactctgaagatccggtccacaaagctggaggactcagccatgtacttctgtgccagcagtgagggacagtactcctacgagcagtacttcgggccgggcaccaggctcacggtcaca

SEQ ID NO: 13 - protein, 9 aa, Homo sapiens
VVGAGGVGK

SEQ ID NO: 14 - protein, 10 aa, Homo sapiens
VVVGAGGVGK

SEQ ID NO: 15 - protein, 9 aa, Homo sapiens
VVGAVGVGK

SEQ ID NO: 16 - protein, 10 aa, Homo sapiens
VVVGAVGVGK

SEQ ID NO: 17 - DNA, 411 bp, Mus musculus
  source 1..411: mol_type = genomic DNA
aacatccagaatccagagcctgccgtgtaccagctgaaggacccacggagccaggatagcaccctgtgcctgttcacagactttgattctcagatcaatgtgcctaagacaatggagagcggcaccttcatcacagacaagtgcgtgctggatatgaaggctatggactctaagagcaacggcgccatcgcctggtccaatcagacctctttcacatgccaggatatctttaaggagacaaacgccacatacccttctagcgacgtgccatgtgatgccaccctgacagagaagtccttcgagacagacatgaacctgaattttcagaacctgctggtcatcgtgctgaggatcctgctgctgaaggtggccggcttcaatctgctgatgaccctgcgcctgtggtcctct

SEQ ID NO: 18 - DNA, 519 bp, Mus musculus
  source 1..519: mol_type = genomic DNA
gaggacctgagaaacgtgacaccccctaaggtgtccctgttcgagccctctaaggccgagatcgccaataagcagaaggccaccctggtgtgcctggccagaggcttctttcctgatcacgtggagctgtcctggtgggtgaacggcaaggaggtgcactctggcgtgtgcaccgacccacaggcctacaaggagagcaattactcctattgtctgtctagccggctgagagtgtccgccacattttggcacaaccctaggaatcacttccgctgccaggtgcagtttcacggcctgtctgaggaggataagtggccagagggaagcccaaagcctgtgacccagaacatctccgccgaggcatggggaagggcagactgtggcatcacctccgcctcttatcagcagggcgtgctgagcgccacaatcctgtacgagatcctgctgggcaaggccaccctgtatgccgtgctggtgagcacactggtggtcatggctatggtgaagagaaagaacagc

SEQ ID NO: 19 - protein, 119 aa, Homo sapiens
AQSVAQPEDQVNVAEGNPLTVKCTYSVSGNPYLFWYVQYPNRGLQFLLKYITGDNLVKGSYGFEAEFNKSQTSFHLKKPSALVSDSALYFCAVRDIEGAGNNRKLIWGLGTSLAVNPNI

SEQ ID NO: 20 - protein, 116 aa, Homo sapiens
EPEVTQTPSHQVTQMGQEVILRCVPISNHLYFYWYRQILGQKVEFLVSFYNNEISEKSEIFDDQFSVERPDGSNFTLKIRSTKLEDSAMYFCASSEGQYSYEQYFGPGTRLTVTED

SEQ ID NO: 21 - protein, 251 aa, Mus musculus
AIQMTQSPSSLSASVGDRVTITCRASQDIRNYLNWYQQKPGKAPKLLIYYTSRLESGVPSRFSGSGSGTDYTLTISSLQPEDFATYYCQQGNTLPWTFGQGTKVEIKGGGGSGGGGSGGGGSGGGGSGGGSEVQLVESGGGLVQPGGSLRLSCAASGYSFTGYTMNWVRQAPGKGLEWVALINPYKGVSTYNQKFKDRFTISVDKSKNTAYLQMNSLRAEDTAVYYCARSGYYGDSDWYFDVWGQGTLVTV

SEQ ID NO: 22 - protein, 7 aa, synthetic construct
  REGION 1..7: note = linker
SSGGGGS

SEQ ID NO: 23 - DNA, 357 bp, synthetic construct
  misc_feature 1..357: note = Coding sequence of a modifiedo alpha chain variable region
  source 1..357: mol_type = other DNA
gctcagtctgttgctcagccggaagaccaggttaacgttgctgaaggtaacccgctgaccgttaaatgcacctactctgtttctggtaacccgtacctgttctggtacgttcagtacccgaaccgtggtctgcagttcctgctgaaatacatcaccggtgacaacctggttaaaggttcttacggtttcgaagctgaattcaacaaatctcagacctctttccacctgaaaaaaccgtctgctctggtttctgactctgctctgtacttctgcgctgttcgtgacatcgaaggtgctggtaacaaccgtaaactgatctggggtctgggtacctctctggctgttaacccgaacatc

SEQ ID NO: 24 - DNA, 348 bp, synthetic construct
  misc_feature 1..348: note = Coding sequence of modified beta chain variable region
  source 1..348: mol_type = other DNA
gaaccggaagttacccagaccccgtctcaccaggttacccagatgggtcaggaagttatcctgcgttgcgttccgatctctaaccacctgtacttctactggtaccgtcagatcctgggtcagaaagttgaattcctggtttctttctacaacaacgaaatctctgaaaaatctgaaatcttcgacgaccagttctctgttgaacgtccggacggttctaacttcaccctgaaaatccgttctaccaaactggaagactctgctatgtacttctgcgcttcttctgaaggtcagtactcttacgaacagtacttcggtccgggtacccgtctgaccgttaccgaagac

SEQ ID NO: 25 - protein, 27 aa, synthetic construct
  REGION 1..27: note = SGSG-P2A
RAKRSGSGATNFSLLKQAGDVEENPGP

SEQ ID NO: 26 - DNA, 81 bp, synthetic construct
  misc_feature 1..81: note = SGSG-P2A
  source 1..81: mol_type = other DNA
cgggccaagagatccggctctggcgccacaaactttagcctgctgaagcaggccggcgatgtggaggagaatcctggccca

SEQ ID NO: 27 - DNA, 19 bp, synthetic construct
  misc_feature 1..19: note = primer
  source 1..19: mol_type = other DNA
aacatccagaatccagagc

SEQ ID NO: 28 - DNA, 20 bp, synthetic construct
  misc_feature 1..20: note = primer
  source 1..20: mol_type = other DNA
cttacacagtcctgctgacc

SEQ ID NO: 29 - DNA, 21 bp, synthetic construct
  misc_feature 1..21: note = primer
  source 1..21: mol_type = other DNA
ctcagttgaaaggcctgatgg

SEQ ID NO: 30 - DNA, 26 bp, synthetic construct
  misc_feature 1..26: note = primer
  source 1..26: mol_type = other DNA
ccgcggtaccgtcgactgcagaattc